European Patent Application EP 4 183 875 A1, published May 24, 2023. Title: improved bioluminescent system. Applicant: Max-Planck-Gesellschaft zur Foerderung der Wissenschaften e.V. The sequence listing filed with the application follows.

SEQUENCE LISTING (29 sequences)

SEQ ID NO: 1 - DNA, 1443 bp, P. luminescens
  CDS (1)..(1443)
atgactaaaaaaatttcattcattattaacggccaggttgaaatctttcccgaaagtgatgatttagtgcaatccattaattttggtgataatagtgtttacctgccaatattgaatgactctcatgtaaaaaacattattgattgtaatggaaataacgaattacggttgcataacattgtcaattttctctatacggtagggcaaagatggaaaaatgaagaatactcaagacgcaggacatacattcgtgacttaaaaaaatatatgggatattcagaagaaatggctaagctagaggccaattggatatctatgattttatgttctaaaggcggcctttatgatgttgtagaaaatgaacttggttctcgccatatcatggatgaatggctacctcaggatgaaagttatgttcgggcttttccgaaaggtaaatctgtacatctgttggcaggtaatgttccattatctgggatcatgtctatattacgcgcaattttaactaagaatcagtgtattataaaaacatcgtcaaccgatccttttaccgctaatgcattagcgttaagttttattgatgtagaccctaatcatccgataacgcgctctttatctgttatatattggccccaccaaggtgatacatcactcgcaaaagaaattatgcgacatgcggatgttattgtcgcttggggagggccagatgcgattaattgggcggtagagcatgcgccatcttatgctgatgtgattaaatttggttctaaaaagagtctttgcattatcgataatcctgttgatttgacgtccgcagcgacaggtgcggctcatgatgtttgtttttacgatcagcgagcttgtttttctgcccaaaacatatattacatgggaaatcattatgaggaatttaagttagcgttgatagaaaaacttaatctatatgcgcatatattaccgaatgccaaaaaagattttgatgaaaaggcggcctattctttagttcaaaaagaaagcttgtttgctggattaaaagtagaggtggatattcatcaacgttggatgattattgagtcaaatgcaggtgtggaatttaatcaaccacttggcagatgtgtgtaccttcatcacgtcgataatattgagcaaatattgccttatgttcaaaaaaataagacgcaaaccatatctatttttccttgggagtcatcatttaaatatcgagatgcgttagcattaaaaggtgcggaaaggattgtagaagcaggaatgaataacatatttcgagttggtggatctcatgacggaatgagaccgttgcaacgattagtgacatatatttctcatgaaaggccatctaactatacggctaaggatgttgcggttgaaatagaacagactcgattcctggaagaagataagttccttgtatttgtcccataa

SEQ ID NO: 2 - protein, 480 aa, P. luminescens
MTKKISFIINGQVEIFPESDDLVQSINFGDNSVYLPILNDSHVKNIIDCNGNNELRLHNIVNFLYTVGQRWKNEEYSRRRTYIRDLKKYMGYSEEMAKLEANWISMILCSKGGLYDVVENELGSRHIMDEWLPQDESYVRAFPKGKSVHLLAGNVPLSGIMSILRAILTKNQCIIKTSSTDPFTANALALSFIDVDPNHPITRSLSVIYWPHQGDTSLAKEIMRHADVIVAWGGPDAINWAVEHAPSYADVIKFGSKKSLCIIDNPVDLTSAATGAAHDVCFYDQRACFSAQNIYYMGNHYEEFKLALIEKLNLYAHILPNAKKDFDEKAAYSLVQKESLFAGLKVEVDIHQRWMIIESNAGVEFNQPLGRCVYLHHVDNIEQILPYVQKNKTQTISIFPWESSFKYRDALALKGAERIVEAGMNNIFRVGGSHDGMRPLQRLVTYISHERPSNYTAKDVAVEIEQTRFLEEDKFLVFVP

SEQ ID NO: 3 - DNA, 1443 bp, artificial sedquence
  mutated LuxC from P. luminescens
  CDS (1)..(1443)
atgactaaaaaaatttcattcattattaccggccaggttgaaatctttcccgaaagcgatgatttagtgcaatccattaattttggtgataatagtgtttacctgccaatattgaatgactctcatgtaaaaaacattattgattgtaatggaaataacgaattacggttgcatgacattgtcaattttctctatacggtagggcaaagatggaaaaatgatgaatactcaagacgcaggacatacattcgtgacttaaaaaaatatatgggatattcagaagaaatggctaagctagaggccaattggatatctatgatattatgttctaaaggcggcctttatgatgttgtagaaaatgaacttggttctcgccatatcatggatgaatggctacctcaggatgaaagttatgttcgggcttttccgaaaggtaaatctgtacatctgttggcaggtaatgttccattatctgggatcatgtctatattacgcgcaattttaactaagaatcagtgtattataaaaacatcgtcaaccgatccttttaccgctaatgcattagcgttaagttttattgatgtagaccctaatcatccgataacgcgctctttatctgttatatattggccccaccaaggtgatacatcactcgcaaaagaaattatgcgacatgcggatgttattgtcgcttggggagggccagatgcgattaattgggcggtagagcatgcgccatcttatgctgatgtgattaaatttggtcctaaaaagagtctttgcattatcgataatcctgttgatttgacgtctgcagcgacaggtgcggctcatgatgtttgtttttacgatcagcgagcttgtttttctgcccaaaacatatattatatgggaaatcattatgaggaatttaagttagcgttgatagaaaaacttaatctatatgcgcatatattaccgaatgcaaaaaaagattttgatgaaaaggcggcctattctttagttcaaaaagaaagcttgtttgctggattaaaagtagaggtggatattcatcaacgttggacgattattgagtcagatgcaggtgtggaatttaatcaaccacttggcagatgtgtgtaccttcatcacgtcgataatattgagcaaatattgccttatgttcaaaaaaataagacgcaaaccatatctatttttccttgggagtcatcatttaaatatcgagatgcgttagcattaaaaggtgcggaaaggattgtagaagcaggaatgaataacatatttcgagttggtggatctcatgacggaatgagaccgttgcaacgattagtgacatatatttctcatgaaaggccatctaactatacggctaaggatgttgcggttgaaatagaacagactcgtttcctggaagaagataagttccttgtatttgtcccataa

SEQ ID NO: 4 - protein, 480 aa, artificial sedquence
  Synthetic Construct
MTKKISFIITGQVEIFPESDDLVQSINFGDNSVYLPILNDSHVKNIIDCNGNNELRLHDIVNFLYTVGQRWKNDEYSRRRTYIRDLKKYMGYSEEMAKLEANWISMILCSKGGLYDVVENELGSRHIMDEWLPQDESYVRAFPKGKSVHLLAGNVPLSGIMSILRAILTKNQCIIKTSSTDPFTANALALSFIDVDPNHPITRSLSVIYWPHQGDTSLAKEIMRHADVIVAWGGPDAINWAVEHAPSYADVIKFGPKKSLCIIDNPVDLTSAATGAAHDVCFYDQRACFSAQNIYYMGNHYEEFKLALIEKLNLYAHILPNAKKDFDEKAAYSLVQKESLFAGLKVEVDIHQRWTIIESDAGVEFNQPLGRCVYLHHVDNIEQILPYVQKNKTQTISIFPWESSFKYRDALALKGAERIVEAGMNNIFRVGGSHDGMRPLQRLVTYISHERPSNYTAKDVAVEIEQTRFLEEDKFLVFVP

SEQ ID NO: 5 - DNA, 924 bp, P. luminescens
  CDS (1)..(921)
atggaaaatgaatcaaaatataaaaccatcgaccacgttatttgtgttgaaggaaataaaaaaattcatgtttgggaaacgctgccagaagaaaacagcccaaagagaaagaatgccattattattgcgtctggttttgcccgcaggatggatcattttgctggtctggcggaatatttatcgcggaatggatttcatgtgatccgctatgattcgcttcaccacgttggattgagttcagggacaattgatgaatttacaatgtctataggaaagcagagcttgttagcagtggttgattggttaactacacgaaaaataaataacttcggtatgttggcttcaagcttatctgcgcggatagcttatgcaagcctatctgaaatcaatgcttcgtttttaatcaccgcagtcggtgttgttaacttaagatattctcttgaaagagctttagggtttgattatctcagtctacccattaatgaattgccgaataatctagattttgaaggccataaattgggtgctgaagtctttgcgagagattgtcttgattttggttgggaagatttagcttctacaattaataacatgatgtatcttgatataccgtttattgcttttactgcaaataacgataattgggtcaagcaagatgaagttatcacattgttatcaaatattcgtagtaatcgatgcaagatatattctttgttaggaagttcgcatgacttgagtgaaaatttagtggtcctgcgcaatttttatcaatcggttacgaaagccgctatcgcgatggataatgatcatctggatattgatgttgatattactgaaccgtcatttgaacatttaactattgcgacagtcaatgaacgccgaatgagaattgagattgaaaatcaagcaatttctctgtcttaa

SEQ ID NO: 6 - protein, 307 aa, P. luminescens
MENESKYKTIDHVICVEGNKKIHVWETLPEENSPKRKNAIIIASGFARRMDHFAGLAEYLSRNGFHVIRYDSLHHVGLSSGTIDEFTMSIGKQSLLAVVDWLTTRKINNFGMLASSLSARIAYASLSEINASFLITAVGVVNLRYSLERALGFDYLSLPINELPNNLDFEGHKLGAEVFARDCLDFGWEDLASTINNMMYLDIPFIAFTANNDNWVKQDEVITLLSNIRSNRCKIYSLLGSSHDLSENLVVLRNFYQSVTKAAIAMDNDHLDIDVDITEPSFEHLTIATVNERRMRIEIENQAISLS

SEQ ID NO: 7 - DNA, 924 bp, artificial sequence; identical to SEQ ID NO: 5
  mutated luxD P. luminescens
  CDS (1)..(924)

SEQ ID NO: 8 - protein, 307 aa, artificial sequence; identical to SEQ ID NO: 6
  Synthetic Construct

SEQ ID NO: 9 - DNA, 1113 bp, P. luminescens
  CDS (1)..(1113)
atgacttcatatgttgataaacaagaaattacagcaagctcagaaattgatgatttgattttttcgagcgatccattagtgtggtcttacgacgagcaggaaaaaatcagaaagaaacttgtgcttgatgcatttcgtaatcattataaacattgtcgagaatatcgtcactactgtcaggcacacaaagtagatgacaatattacggaaattgatgacatacctgtattcccaacatcggtttttaagtttactcgcttattaacttctcaggaaaacgagattgaaagttggtttaccagtagcggcacgaatggtttaaaaagtcaggtggcgcgtgacagattaagtattgagagactcttaggctctgtgagttatggcatgaaatatgttggtagttggtttgatcatcaaatagaattagtcaatttgggaccagatagatttaatgctcataatatttggtttaaatatgttatgagtttggtggaattgttatatcctacgacatttaccgtaacagaagaacgaatagattttgttaaaacattgaatagtcttgaacgaataaaaaatcaagggaaagatctttgtcttattggttcgccatactttatttatttactctgccattatatgaaagataaaaaaatctcattttctggagataaaagcctttatatcataaccggaggcggctggaaaagttacgaaaaagaatctctgaaacgtgatgatttcaatcatcttttatttgatactttcaatctcagtgatattagtcagatccgagatatatttaatcaagttgaactcaacacttgtttctttgaggatgaaatgcagcgtaaacatgttccgccgtgggtatatgcgcgagcgcttgatcctgaaacgttgaaacctgtacctgatggaacgccggggttgatgagttatatggatgcgtcagcaaccagttatccagcatttattgttaccgatgatgtcgggataattagcagagaatatggtaagtatcccggcgtgctcgttgaaattttacgtcgcgtcaatacgaggacgcagaaagggtgtgctttaagcttaaccgaagcgtttgatagttga

SEQ ID NO: 10 - protein, 370 aa, P. luminescens
MTSYVDKQEITASSEIDDLIFSSDPLVWSYDEQEKIRKKLVLDAFRNHYKHCREYRHYCQAHKVDDNITEIDDIPVFPTSVFKFTRLLTSQENEIESWFTSSGTNGLKSQVARDRLSIERLLGSVSYGMKYVGSWFDHQIELVNLGPDRFNAHNIWFKYVMSLVELLYPTTFTVTEERIDFVKTLNSLERIKNQGKDLCLIGSPYFIYLLCHYMKDKKISFSGDKSLYIITGGGWKSYEKESLKRDDFNHLLFDTFNLSDISQIRDIFNQVELNTCFFEDEMQRKHVPPWVYARALDPETLKPVPDGTPGLMSYMDASATSYPAFIVTDDVGIISREYGKYPGVLVEILRRVNTRTQKGCALSLTEAFDS

SEQ ID NO: 11 - DNA, 1083 bp, artificial sequence
  mutated luxA of P.luminescens
  CDS (1)..(1083)
atgaaatttggaaactttttacttacataccaacctccccaattttctcaaacagaggtaatggaacgtttggttaaattaggtcgcatctctgaggagtgtggttttgataccgtatggttactggagcatcatttcacggagtttggtctacttggtaacccttatgtcgctgctgcatatttacttggcgcgactaaaaaattgaatgtaggaaccgccgctattgttcttcccacagcccatccagtacgccaacttgaagatgtgaatttattggatcaaatgtcaaaaggacgatttcggtttggtatttgccgagggctttacaacaaggactttcgcgtattcggcgcggatatgaataacagtcgcgccttagcggaatgctggtacgggctgataaagaatggcatgacagagggatatatggaagctgataatgaacatatcaagttccataaggtaaaagtaaaccccgcggcgtatagcagaggtggcgcaccggtttatgtggtggctgaatcagctgcgacgactgagtgggcagctcaatttggcctaccgatgatattaagttggattataaatactaacgaaaagaaagcacaacttgagctttataatgaggtggctcaagaatatgggcacgatattcataatatcgaccattgcttatcatatataacatctgtagatcatgactcaattaaagcgaaagagatttgccggaaatttctggggcattggtatgattcttatgtgaatgctacgactatttttgatgattcagaccaaacaagaggttatgatttcaataaagggcagtggcgtgactttgtattaaaaggacataaagatactaatcgccgtattgattacagttacgaaatcaatcccgtgggaacgccgcaggaatgtattgacataattcaaaaagacattgatgctacaggaatatcaaatatttgttgtggatttgaagctaatggaacagtagacgaaattattgcttccatgaagctcttccagtctgatgtcatgccatttcttaaagaaaaacaacgttcgctattatattag

SEQ ID NO: 12 - protein, 360 aa, artificial sequence
  Synthetic Construct
MKFGNFLLTYQPPQFSQTEVMERLVKLGRISEECGFDTVWLLEHHFTEFGLLGNPYVAAAYLLGATKKLNVGTAAIVLPTAHPVRQLEDVNLLDQMSKGRFRFGICRGLYNKDFRVFGADMNNSRALAECWYGLIKNGMTEGYMEADNEHIKFHKVKVNPAAYSRGGAPVYVVAESAATTEWAAQFGLPMILSWIINTNEKKAQLELYNEVAQEYGHDIHNIDHCLSYITSVDHDSIKAKEICRKFLGHWYDSYVNATTIFDDSDQTRGYDFNKGQWRDFVLKGHKDTNRRIDYSYEINPVGTPQECIDIIQKDIDATGISNICCGFEANGTVDEIIASMKLFQSDVMPFLKEKQRSLLY

SEQ ID NO: 13 - DNA, 984 bp, artificial sequence
  mutated luxB of P. luminescens
  CDS (1)..(984)
atgaaatttggattgttcttccttaacttcatcaatccgacaactgttcaagaacaaagtatagttcgcatgcaggaaataacggagtatgttgataagttgaattttgaacagattttagtgtatgaaaatcatttttcagataatggtgttgtcggcgctcctctgactgtttctggttttctgctcggtttaacagagaaaattaaaattggttcattaaatcacatcattacaactcatcatcctgtccgcatagcggaggaagcttgcttattggatcagttaagtgaagggagatttattttagggtttagtgattgcgaaaaaaaagatgaaatgcatttttttaatcgcccggctgaatatcaacagcaactatttgaagagtgttatgaaatcattaacgatgctttaacaacaggctattgtaatccagataacgatttttatagcttccctaaaatatctgtaaatccccatgcttatacgccaggcggacctcggaaatatgtaacagcaaccagtcatcatattgttgagtgggcggccaaaaaaggtattcctctcatctttaagtgggatgattctaatgatgttagatatgaatatgctgaaagatataaagccgtcgcggataaatatgacgttgacctatcagagatagaccatcagttaatgatattagttaactataacgaagatagtaataaagctaaacaagagacgcgtgcatttattagtgattatgttcttgaaatgcaccctaatgaagatttcgaaaataaacttgaagaaataattgcagaaaacgctgtcggaaattatacggagtgtataactgcggctaaattggcaattgaaaagtgtggtgcgaaaagtgtattgctgtcctttgaaccaatgaatgatttgatgagccaaaaaaatgtaatcaatattgttgatgataatattaagaagtaccacatggaatatacctaa

SEQ ID NO: 14 - protein, 327 aa, artificial sequence
  Synthetic Construct
MKFGLFFLNFINPTTVQEQSIVRMQEITEYVDKLNFEQILVYENHFSDNGVVGAPLTVSGFLLGLTEKIKIGSLNHIITTHHPVRIAEEACLLDQLSEGRFILGFSDCEKKDEMHFFNRPAEYQQQLFEECYEIINDALTTGYCNPDNDFYSFPKISVNPHAYTPGGPRKYVTATSHHIVEWAAKKGIPLIFKWDDSNDVRYEYAERYKAVADKYDVDLSEIDHQLMILVNYNEDSNKAKQETRAFISDYVLEMHPNEDFENKLEEIIAENAVGNYTECITAAKLAIEKCGAKSVLLSFEPMNDLMSQKNVINIVDDNIKKYHMEYT

SEQ ID NO: 15 - DNA, 774 bp, artificial sequence
  mutated frp from Vibrio campbellii
  CDS (1)..(774)
atggtgaagatacagcccatccccacaactagccagggcagcctttttataatgaatagcaccatagagacaatcctgggccatagatccattaggaagttcacatctgaacctattgctagtgagcagctgcaaacgattcttcagtctgggctcgctgcttcaagctcatccatgctgcaggttgtgagtataattcgggttacagacacggaaaagagaaaattgctcgctcaatatgccggcaaccagacgtatgtggaatccgctgctgagttcctggtcttttgtatagactaccagcgacacgctactatcaaccccgatgtccaagctgactttaccgagctgaccctgattggtgcagtggattccggcataatggcccagaattgcctcctggcagcagaatcaatgggtcttggcggagtctatatcggaggacttcggaactcagctgcccaagtggatgagttgctcggactgcccaagaacacagctatcctcttcggaatgtgcttggggcaccccgatcagagccctgagacaaagcctagactgcccgctcatgtgatcgtgcacgagaaccaatatcaagctctgaacattgacgacgtacaggcgtatgacaaaacattgcaggagtattatgccagcagaaccagcaaccagaagcagagtgtctggtcccaggaaactgcaggcaagctggccggagaatccctcccacacatcctgccatacctgaactccaagggccttgccagaaggtaa

SEQ ID NO: 16 - protein, 257 aa, artificial sequence
  Synthetic Construct
MVKIQPIPTTSQGSLFIMNSTIETILGHRSIRKFTSEPIASEQLQTILQSGLAASSSSMLQVVSIIRVTDTEKRKLLAQYAGNQTYVESAAEFLVFCIDYQRHATINPDVQADFTELTLIGAVDSGIMAQNCLLAAESMGLGGVYIGGLRNSAAQVDELLGLPKNTAILFGMCLGHPDQSPETKPRLPAHVIVHENQYQALNIDDVQAYDKTLQEYYASRTSNQKQSVWSQETAGKLAGESLPHILPYLNSKGLARR

SEQ ID NO: 17 - DNA, 6605 bp, artificial sequence
  operon ilux 2
atgactaaaaaaatttcattcattattaatggccaggtagaaatctttcccgaaagcgatgatttagtgcaatccatcacttttggtgataatagtgtttacctgccaatattgaacgactctcatgtaaaaaccattactgattgtaatggaaataacgacttacggttgcatgacattgtcaattttctctatacggtagggcaaagatggaaaaataatgaatacccaagacgcaggacatacattcgtgacttaaaaaaatatatgggatattcagaagaaatggctaagctagaggccaattggatatctatgatattatgttctaaaggcggcctttatgatgttgtagaaaatgaacttggttctcgccatatcatggatgaatggatacctcagggtgaaagttatgttcgggcttttccgaaaggtaaatccgtacatctgttggcaggtaatgttccattatctgggatcatgtctatattacgtgcaattttaactaagaatcagtgtattataaaaacatcgtcaaccgatccttttaccgctaatgcattagctttaagttttattgatgtagaccctaatcatccgataacgcgctctttatctgttatatattggccccaccaaggtgatatatcactcgcaaaagaaattatgcgacatgcggatgttattgtcgcatggggagggccagatgcgattaattgggcggtagagcatgcgccatctaatgctgatgtgattaaatttggtcctaaaaagagcctttgcattatcgataatcctgttgatctgacgtctgcagcgacaggtgcggctcatgatgtttgtttttacgatcagcgagcttgcttttctgcccaaaacatatattatatgggaaatcattatgaggaatttaagttggcattgatagaaaaacttaatctatatgcgcatatattaccgaatgcaaaaaaagattttgatgaaaaggcggcctattctttagttcaaaaagagagcttgtttgccggattaaatgtagaggcggatattcatcaacgttggacgattattgagtcagatgcaggtgtggaatttaatcaaccacttggcagatgtgtgtaccttcatcacgtcgataatattgagcaaatattgccttatgttcaaaaaaataagacgcaaaccatatctatttttccttgggagtcatcatttaaatatcgagatgcgttagcattagaaggtgcggaaaggattgtagaagcaggaatgaataacatatttcgagttggtggatctcatgacggaatgagaccgttgcaacgattagtgaagtatatttctcatgaaaggccatctaactatacggctaaggatgttgcggttgaaatagaacagactcgtttcctggaagaagacaagttccttgtatttgtcccataataggtaaaaagtatggaaaaagaatcaaaatataaaaccatcgaccacgttatttgtgttgaaggaaataaaaaaattcatgtttgggaaacgctgccagaagaaaacagcccaaagagaaagaatgccattattattgcgtctggttttgcccgcaggatggatcattttgctggactggcggaatatttatcgcggaatgggtttcatgtgatccgctatgattcgcttcaccacgttggattgagttcagggacaattgatgaatttacaatgtctacaggaaagcagagcttgttagcagtggttgattggttaactacacgaaatataagtaacttcggtgtgttggcttcaagcttatctgcgcggatagcttatgcaagcctatctgaaatcaatgcttcgtttttaatcaccgcagtcggtgttgttaacttaagatattctcttgaaagagctttagggtttgattatctcagtcttcccattaatgaattgccgaaaaatctagtttttgaaggccataaattgggtgctgaagtcttcgcgagagattgtcttgattttggttgggaagacttagcttctacaattaataacatgatgtatcttgatataccgtttattgcttttaccgcaaataacgacaattgggtcaagcaagatgaagttatcacattgttatcaaatattcgaagtaatcgatgtaggatatattctttgttaggaagttcgcatgacttgagtgaaaatttagtggccctgcgcaatttttatcaatcggttacgaaagccgctatcgcgatggataatgatcatctggatattaatgttgatattactgaaccgtcatttgaacatttaactattgcgacagtcaatgaacgccgaatgagaattgagattgtaaatcaagcaatttctctgtcttaaaatctattgagatattctatcactcaaatagcaatataaggactctctgaattcatgaaatttggaaactttttacttacataccaacctccccaattttctcaaacagaggtaatggaacgtttggttaaattaggtcgcatctctgaggagtgtggttttgataccgtatggttactggagcatcatttcacggagtttggtctacttggtaacccttatgtcgctgctgcatatttacttggcgcgactaaaaaattgaatgtaggaaccgccgctattgttcttcccacagcccatccagtacgccaacttgaagatgtgaatttattggatcaaatgtcaaaaggacgatttcggtttggtatttgccgagggctttacaacaaggactttcgcgtattcggcgcggatatgaataacagtcgcgccttagcggaatgctggtacgggctgataaagaatggcatgacagagggatatatggaagctgataatgaacatatcaagttccataaggtaaaagtaaaccccgcggcgtatagcagaggtggcgcaccggtttatgtggtggctgaatcagctgcgacgactgagtgggcagctcaatttggcctaccgatgatattaagttggattataaatactaacgaaaagaaagcacaacttgagctttataatgaggtggctcaagaatatgggcacgatattcataatatcgaccattgcttatcatatataacatctgtagatcatgactcaattaaagcgaaagagatttgccggaaatttctggggcattggtatgattcttatgtgaatgctacgactatttttgatgattcagaccaaacaagaggttatgatttcaataaagggcagtggcgtgactttgtattaaaaggacataaagatactaatcgccgtattgattacagttacgaaatcaatcccgtgggaacgccgcaggaatgtattgacataattcaaaaagacattgatgctacaggaatatcaaatatttgttgtggatttgaagctaatggaacagtagacgaaattattgcttccatgaagctcttccagtctgatgtcatgccatttcttaaagaaaaacaacgttcgctattatattagctaaggagaaagaaatgaaatttggattgttcttccttaacttcatcaatccgacaactgttcaagaacaaagtatagttcgcatgcaggaaataacggagtatgttgataagttgaattttgaacagattttagtgtatgaaaatcatttttcagataatggtgttgtcggcgctcctctgactgtttctggttttctgctcggtttaacagagaaaattaaaattggttcattaaatcacatcattacaactcatcatcctgtccgcatagcggaggaagcttgcttattggatcagttaagtgaagggagatttattttagggtttagtgattgcgaaaaaaaagatgaaatgcatttttttaatcgcccggctgaatatcaacagcaactatttgaagagtgttatgaaatcattaacgatgctttaacaacaggctattgtaatccagataacgatttttatagcttccctaaaatatctgtaaatccccatgcttatacgccaggcggacctcggaaatatgtaacagcaaccagtcatcatattgttgagtgggcggccaaaaaaggtattcctctcatctttaagtgggatgattctaatgatgttagatatgaatatgctgaaagatataaagccgtcgcggataaatatgacgttgacctatcagagatagaccatcagttaatgatattagttaactataacgaagatagtaataaagctaaacaagagacgcgtgcatttattagtgattatgttcttgaaatgcaccctaatgaagatttcgaaaataaacttgaagaaataattgcagaaaacgctgtcggaaattatacggagtgtataactgcggctaaattggcaattgaaaagtgtggtgcgaaaagtgtattgctgtcctttgaaccaatgaatgatttgatgagccaaaaaaatgtaatcaatattgttgatgataatattaagaagtaccacatggaatatacctaaccatggtagatttcgagttgcagcgaggcggcaagtgaacgaatccccaggagcatagataactatgtgactggggtgagtgaaagcagccaacaaagcagcagcttgaaagatgaagggtataaaagagtatgacagcagtgctgccatactttctaatattatcttgaggagtaaaacaggtatgacttcatatgttgataaacaagaaattacagcaagctcagaaattgatgatttgattttttcgagcgatccattagtgtggtcttacgacgagcaggaaaaaatcagaaagaaacttgtgcttgatgcatttcgtaatcattataaacattgtcgagaatatcgtcactactgtcaggcacacaaagtagatgacaatattacggaaattgatgacatacctgtattcccaacatcggtttttaagtttactcgcttattaacttctcaggaaaacgagattgaaagttggtttaccagtagcggcacgaatggtttaaaaagtcaggtggcgcgtgacagattaagtattgagagactcttaggctctgtgagttatggcatgaaatatgttggtagttggtttgatcatcaaatagaattagtcaatttgggaccagatagatttaatgctcataatatttggtttaaatatgttatgagtttggtggaattgttatatcctacgacatttaccgtaacagaagaacgaatagattttgttaaaacattgaatagtcttgaacgaataaaaaatcaagggaaagatctttgtcttattggttcgccatactttatttatttactctgccattatatgaaagataaaaaaatctcattttctggagataaaagcctttatatcataaccggaggcggctggaaaagttacgaaaaagaatctctgaaacgtgatgatttcaatcatcttttatttgatactttcaatctcagtgatattagtcagatccgagatatatttaatcaagttgaactcaacacttgtttctttgaggatgaaatgcagcgtaaacatgttccgccgtgggtatatgcgcgagcgcttgatcctgaaacgttgaaacctgtacctgatggaacgccggggttgatgagttatatggatgcgtcagcaaccagttatccagcatttattgttaccgatgatgtcgggataattagcagagaatatggtaagtatcccggcgtgctcgttgaaattttacgtcgcgtcaatacgaggacgcagaaagggtgtgctttaagcttaaccgaagcgtttgatagttgagtcgacctaaggagaaagaaatggtgaagatacagcccatccccacaactagccagggcagcctttttataatgaatagcaccatagagacaatcctgggccatagatccattaggaagttcacatctgaacctattgctagtgagcagctgcaaacgattcttcagtctgggctcgctgcttcaagctcatccatgctgcaggttgtgagtataattcgggttacagacacggaaaagagaaaattgctcgctcaatatgccggcaaccagacgtatgtggaatccgctgctgagttcctggtcttttgtatagactaccagcgacacgctactatcaaccccgatgtccaagctgactttaccgagctgaccctgattggtgcagtggattccggcataatggcccagaattgcctcctggcagcagaatcaatgggtcttggcggagtctatatcggaggacttcggaactcagctgcccaagtggatgagttgctcggactgcccaagaacacagctatcctcttcggaatgtgcttggggcaccccgatcagagccctgagacaaagcctagactgcccgctcatgtgatcgtgcacgagaaccaatatcaagctctgaacattgacgacgtacaggcgtatgacaaaacattgcaggagtattatgccagcagaaccagcaaccagaagcagagtgtctggtcccaggaaactgcaggcaagctggccggagaatccctcccacacatcctgccatacctgaactccaagggccttgccagaaggtaa

SEQ ID NO: 18 - DNA, 1443 bp, artificial sequence
  mutated luxC of P. luminescens
  CDS (1)..(1443)
atgactaaaaaaatttcattcattattaatggccaggtagaaatctttcccgaaagcgatgatttagtgcaatccatcacttttggtgataatagtgtttacctgccaatattgaacgactctcatgtaaaaaccattactgattgtaatggaaataacgacttacggttgcatgacattgtcaattttctctatacggtagggcaaagatggaaaaataatgaatacccaagacgcaggacatacattcgtgacttaaaaaaatatatgggatattcagaagaaatggctaagctagaggccaattggatatctatgatattatgttctaaaggcggcctttatgatgttgtagaaaatgaacttggttctcgccatatcatggatgaatggatacctcagggtgaaagttatgttcgggcttttccgaaaggtaaatccgtacatctgttggcaggtaatgttccattatctgggatcatgtctatattacgtgcaattttaactaagaatcagtgtattataaaaacatcgtcaaccgatccttttaccgctaatgcattagctttaagttttattgatgtagaccctaatcatccgataacgcgctctttatctgttatatattggccccaccaaggtgatatatcactcgcaaaagaaattatgcgacatgcggatgttattgtcgcatggggagggccagatgcgattaattgggcggtagagcatgcgccatctaatgctgatgtgattaaatttggtcctaaaaagagcctttgcattatcgataatcctgttgatctgacgtctgcagcgacaggtgcggctcatgatgtttgtttttacgatcagcgagcttgcttttctgcccaaaacatatattatatgggaaatcattatgaggaatttaagttggcattgatagaaaaacttaatctatatgcgcatatattaccgaatgcaaaaaaagattttgatgaaaaggcggcctattctttagttcaaaaagagagcttgtttgccggattaaatgtagaggcggatattcatcaacgttggacgattattgagtcagatgcaggtgtggaatttaatcaaccacttggcagatgtgtgtaccttcatcacgtcgataatattgagcaaatattgccttatgttcaaaaaaataagacgcaaaccatatctatttttccttgggagtcatcatttaaatatcgagatgcgttagcattagaaggtgcggaaaggattgtagaagcaggaatgaataacatatttcgagttggtggatctcatgacggaatgagaccgttgcaacgattagtgaagtatatttctcatgaaaggccatctaactatacggctaaggatgttgcggttgaaatagaacagactcgtttcctggaagaagacaagttccttgtatttgtcccataa

SEQ ID NO: 19 - protein, 480 aa, artificial sequence
  Synthetic Construct
MTKKISFIINGQVEIFPESDDLVQSITFGDNSVYLPILNDSHVKTITDCNGNNDLRLHDIVNFLYTVGQRWKNNEYPRRRTYIRDLKKYMGYSEEMAKLEANWISMILCSKGGLYDVVENELGSRHIMDEWIPQGESYVRAFPKGKSVHLLAGNVPLSGIMSILRAILTKNQCIIKTSSTDPFTANALALSFIDVDPNHPITRSLSVIYWPHQGDISLAKEIMRHADVIVAWGGPDAINWAVEHAPSNADVIKFGPKKSLCIIDNPVDLTSAATGAAHDVCFYDQRACFSAQNIYYMGNHYEEFKLALIEKLNLYAHILPNAKKDFDEKAAYSLVQKESLFAGLNVEADIHQRWTIIESDAGVEFNQPLGRCVYLHHVDNIEQILPYVQKNKTQTISIFPWESSFKYRDALALEGAERIVEAGMNNIFRVGGSHDGMRPLQRLVKYISHERPSNYTAKDVAVEIEQTRFLEEDKFLVFVP

SEQ ID NO: 20 - DNA, 924 bp, artificial sequence
  mutated luxD of P. luminescens
  CDS (1)..(924)
atggaaaaagaatcaaaatataaaaccatcgaccacgttatttgtgttgaaggaaataaaaaaattcatgtttgggaaacgctgccagaagaaaacagcccaaagagaaagaatgccattattattgcgtctggttttgcccgcaggatggatcattttgctggactggcggaatatttatcgcggaatgggtttcatgtgatccgctatgattcgcttcaccacgttggattgagttcagggacaattgatgaatttacaatgtctacaggaaagcagagcttgttagcagtggttgattggttaactacacgaaatataagtaacttcggtgtgttggcttcaagcttatctgcgcggatagcttatgcaagcctatctgaaatcaatgcttcgtttttaatcaccgcagtcggtgttgttaacttaagatattctcttgaaagagctttagggtttgattatctcagtcttcccattaatgaattgccgaaaaatctagtttttgaaggccataaattgggtgctgaagtcttcgcgagagattgtcttgattttggttgggaagacttagcttctacaattaataacatgatgtatcttgatataccgtttattgcttttaccgcaaataacgacaattgggtcaagcaagatgaagttatcacattgttatcaaatattcgaagtaatcgatgtaggatatattctttgttaggaagttcgcatgacttgagtgaaaatttagtggccctgcgcaatttttatcaatcggttacgaaagccgctatcgcgatggataatgatcatctggatattaatgttgatattactgaaccgtcatttgaacatttaactattgcgacagtcaatgaacgccgaatgagaattgagattgtaaatcaagcaatttctctgtcttaa

SEQ ID NO: 21 - protein, 307 aa, artificial sequence
  Synthetic Construct
MEKESKYKTIDHVICVEGNKKIHVWETLPEENSPKRKNAIIIASGFARRMDHFAGLAEYLSRNGFHVIRYDSLHHVGLSSGTIDEFTMSTGKQSLLAVVDWLTTRNISNFGVLASSLSARIAYASLSEINASFLITAVGVVNLRYSLERALGFDYLSLPINELPKNLVFEGHKLGAEVFARDCLDFGWEDLASTINNMMYLDIPFIAFTANNDNWVKQDEVITLLSNIRSNRCRIYSLLGSSHDLSENLVALRNFYQSVTKAAIAMDNDHLDINVDITEPSFEHLTIATVNERRMRIEIVNQAISLS

SEQ ID NO: 22 - DNA, 1083 bp, P. luminescens
  CDS (1)..(1083)
atgaaatttggaaactttttgcttacataccaacctccccaattttctcaaacagaggtaatgaaacgtttggttaaattaggtcgcatctctgaggagtgtggttttgataccgtatggttactggagcatcatttcacggagtttggtttgcttggtaacccttatgtcgctgctgcatatttacttggcgcgactaaaaaattgaatgtaggaactgccgctattgttcttcccacagcccatccagtacgccaacttgaagatgtgaatttattggatcaaatgtcaaaaggacgatttcggtttggtatttgccgagggctttacaacaaggactttcgcgtattcggcacagatatgaataacagtcgcgccttagcggaatgctggtacgggctgataaagaatggcatgacagagggatatatggaagctgataatgaacatatcaagttccataaggtaaaagtaaaccccgcggcgtatagcagaggtggcgcaccggtttatgtggtggctgaatcagcttcgacgactgagtgggctgctcaatttggcctaccgatgatattaagttggattataaatactaacgaaaagaaagcacaacttgagctttataatgaagtggctcaagaatatgggcacgatattcataatatcgaccattgcttatcatatataacatctgtagatcatgactcaattaaagcgaaagagatttgccggaaatttctggggcattggtatgattcttatgtgaatgctacgactatttttgatgattcagaccaaacaagaggttatgatttcaataaagggcagtggcgtgactttgtattaaaaggacataaagatactaatcgccgtattgattacagttacgaaatcaatcccgtgggaacgccgcaggaatgtattgacataattcaaaaagacattgatgctacaggaatatcaaatatttgttgtggatttgaagctaatggaacagtagacgaaattattgcttccatgaagctcttccagtctgatgtcatgccatttcttaaagaaaaacaacgttcgctattatattag

SEQ ID NO: 23 - protein, 360 aa, P. luminescens
MKFGNFLLTYQPPQFSQTEVMKRLVKLGRISEECGFDTVWLLEHHFTEFGLLGNPYVAAAYLLGATKKLNVGTAAIVLPTAHPVRQLEDVNLLDQMSKGRFRFGICRGLYNKDFRVFGTDMNNSRALAECWYGLIKNGMTEGYMEADNEHIKFHKVKVNPAAYSRGGAPVYVVAESASTTEWAAQFGLPMILSWIINTNEKKAQLELYNEVAQEYGHDIHNIDHCLSYITSVDHDSIKAKEICRKFLGHWYDSYVNATTIFDDSDQTRGYDFNKGQWRDFVLKGHKDTNRRIDYSYEINPVGTPQECIDIIQKDIDATGISNICCGFEANGTVDEIIASMKLFQSDVMPFLKEKQRSLLY

SEQ ID NO: 24 - DNA, 984 bp, P. luminescens
  CDS (1)..(984)
atgaaatttggattgttcttccttaacttcatcaattcaacaactgttcaagaacaaagtatagttcgcatgcaggaaataacggagtatgttgataagttgaattttgaacagattttagtgtatgaaaatcatttttcagataatggtgttgtcggcgctcctctgactgtttctggttttctgctcggtttaacagagaaaattaaaattggttcattaaatcacatcattacaactcatcatcctgtccgcatagcggaggaagcttgcttattggatcagttaagtgaagggagatttattttagggtttagtgattgcgaaaaaaaagatgaaatgcatttttttaatcgcccggttgaatatcaacagcaactatttgaagagtgttatgaaatcattaacgatgctttaacaacaggctattgtaatccagataacgatttttatagcttccctaaaatatctgtaaatccccatgcttatacgccaggcggacctcggaaatatgtaacagcaaccagtcatcatattgttgagtgggcggccaaaaaaggtattcctctcatctttaagtgggatgattctaatgatgttagatatgaatatgctgaaagatataaagccgttgcggataaatatgacgttgacctatcagagatagaccatcagttaatgatattagttaactataacgaagatagtaataaagctaaacaagagacgcgtgcatttattagtgattatgttcttgaaatgcaccctaatgaaaatttcgaaaataaacttgaagaaataattgcagaaaacgctgtcggaaattatacggagtgtataactgcggctaagttggcaattgaaaagtgtggtgcgaaaagtgtattgctgtcctttgaaccaatgaatgatttgatgagccaaaaaaatgtaatcaatattgttgatgataatattaagaagtaccacatggaatatacctaa

SEQ ID NO: 25 - protein, 327 aa, P. luminescens
MKFGLFFLNFINSTTVQEQSIVRMQEITEYVDKLNFEQILVYENHFSDNGVVGAPLTVSGFLLGLTEKIKIGSLNHIITTHHPVRIAEEACLLDQLSEGRFILGFSDCEKKDEMHFFNRPVEYQQQLFEECYEIINDALTTGYCNPDNDFYSFPKISVNPHAYTPGGPRKYVTATSHHIVEWAAKKGIPLIFKWDDSNDVRYEYAERYKAVADKYDVDLSEIDHQLMILVNYNEDSNKAKQETRAFISDYVLEMHPNENFENKLEEIIAENAVGNYTECITAAKLAIEKCGAKSVLLSFEPMNDLMSQKNVINIVDDNIKKYHMEYT

SEQ ID NO: 26 - DNA, 774 bp, Vibrio campbellii
  CDS (1)..(774)
atggtgaagatacagcccatccccacaactagccagggcagcctttttataatgaatagcaccatagagacaatcctgggccatagatccattaggaagttcacatctgaacctattgctagtgagcagctgcaaacgattcttcagtctgggctcgctgcttcaagctcatccatgctgcaggttgtgagtataattcgggttacagacacggaaaagagaaaattgctcgctcaatatgccggcaaccagacgtatgtggaatccgctgctgagttcctggtcttttgtatagactaccagcgacacgctactatcaaccccgatgtccaagctgactttaccgagctgaccctgattggtgcagtggattccggcataatggcccagaattgcctcctggcagcagaatcaatgggtcttggcggagtctatatcggaggacttcggaactcagctgcccaagtggatgagttgctcggactgcccaagaacacagctatcctcttcggaatgtgcttggggcaccccgatcagagccctgagacaaagcctagactgcccgctcatgtgatcgtgcacgagaaccaatatcaagctctgaacattgacgacgtacaggcgtatgacaaaacaatgcaggagtattatgccagcagaaccagcaaccagaagcagagtgtctggtcccaggaaactgcaggcaagctggccggagaatcccgcccacacatcctgccatacctgaactccaagggccttgccaaaaggtaa

SEQ ID NO: 27 - protein, 257 aa, Vibrio campbellii
MVKIQPIPTTSQGSLFIMNSTIETILGHRSIRKFTSEPIASEQLQTILQSGLAASSSSMLQVVSIIRVTDTEKRKLLAQYAGNQTYVESAAEFLVFCIDYQRHATINPDVQADFTELTLIGAVDSGIMAQNCLLAAESMGLGGVYIGGLRNSAAQVDELLGLPKNTAILFGMCLGHPDQSPETKPRLPAHVIVHENQYQALNIDDVQAYDKTMQEYYASRTSNQKQSVWSQETAGKLAGESRPHILPYLNSKGLAKR

SEQ ID NO: 28 - DNA, 20 bp, artificial sequence
  crispr system target sequence
gcggccttttcttttcgtgc

SEQ ID NO: 29 - DNA, 80 bp, artificial sequence
  crispr oligonucleotide
tcatccatcactaccatcaaatactgagcggctcaaaaagaaaaggccgcgtctggcacgatgcggacacgatatacggt